European Patent Application EP 4 273 158 A1, published November 8, 2023. Title: INTERLEUKIN-21 MUTANT AND USE THEREOF. Applicant: Innovent Biologics (Suzhou) Co., Ltd. The sequence listing filed with the application follows.

SEQUENCE LISTING (117 sequences)

SEQ ID NO: 1 - protein, 370 aa, Homo sapiens
  IL-21wt
QGQDRHMIRMRQLIDIVDQLKNYVNDLVPEFLPAPEDVETNCEWSAFSCFQKAQLKSANTGNNERIINVSIKKLKRKPPSTNAGRRQKHRLTCPSCDSYEKKPPKEFLERFKSLLQKMIHQHLSSRTHGSEDSGGGGSGGGGSDKTHTCPPCPAPEAAGGPSVFLFPPKPKDTLMISRTPEVTCVVVDVSHEDPEVKFNWYVDGVEVHNAKTKPREEQYNSTYRVVSVLTVLHQDWLNGKEYKCKVSNKALPAPIEKTISKAKGQPREPQVYTLPPSREEMTKNQVSLTCLVKGFYPSDIAVEWESNGQPENNYKTTPPVLDSDGSFFLYSKLTVDKSRWQQGNVFSCSVMHEALHNHYTQKSLSLSPGK

SEQ ID NO: 2 - protein, 370 aa, Artificial
  Synthetic sequence
HKSDIHMIRMRQLIDIVDQLKNYVNDLVPEFLPAPEDVETNCEWSAFSCFQKAQLKSANTGNNERIINVSIKKLKRKPPSTNAGRRQKHRLTCPSCDSYEKKPPKEFLERFKSLLQKMIHQHLSSRTHGSEDSGGGGSGGGGSDKTHTCPPCPAPEAAGGPSVFLFPPKPKDTLMISRTPEVTCVVVDVSHEDPEVKFNWYVDGVEVHNAKTKPREEQYNSTYRVVSVLTVLHQDWLNGKEYKCKVSNKALPAPIEKTISKAKGQPREPQVYTLPPSREEMTKNQVSLTCLVKGFYPSDIAVEWESNGQPENNYKTTPPVLDSDGSFFLYSKLTVDKSRWQQGNVFSCSVMHEALHNHYTQKSLSLSPGK

SEQ ID NO: 3 - protein, 370 aa, Artificial
  Synthetic sequence
HKCDIHMIRMRQLIDIVDQLKNYVNDLVPEFLPAPEDVETNCEWSAFSCFQKAQLKSANTGNNERIINVSIKKLKRKPPSTNAGRRQKHRLTCPSCDSYEKKPPKEFLERFKSLLQKMIHQHCSSRTHGSEDSGGGGSGGGGSDKTHTCPPCPAPEAAGGPSVFLFPPKPKDTLMISRTPEVTCVVVDVSHEDPEVKFNWYVDGVEVHNAKTKPREEQYNSTYRVVSVLTVLHQDWLNGKEYKCKVSNKALPAPIEKTISKAKGQPREPQVYTLPPSREEMTKNQVSLTCLVKGFYPSDIAVEWESNGQPENNYKTTPPVLDSDGSFFLYSKLTVDKSRWQQGNVFSCSVMHEALHNHYTQKSLSLSPGK

SEQ ID NO: 4 - protein, 370 aa, Artificial
  Synthetic sequence
HKSDITLQEMRQLIDIVDQLKNYVNDLVPEFLPAPEDVETNCEWSAFSCFQKAQLKSANTGNNERIINVSIKKLKRKPPSTNAGRRQKHRLTCPSCDSYEKKPPKEFLERFKSLLQKMIHQHLSSRTHGSEDSGGGGSGGGGSDKTHTCPPCPAPEAAGGPSVFLFPPKPKDTLMISRTPEVTCVVVDVSHEDPEVKFNWYVDGVEVHNAKTKPREEQYNSTYRVVSVLTVLHQDWLNGKEYKCKVSNKALPAPIEKTISKAKGQPREPQVYTLPPSREEMTKNQVSLTCLVKGFYPSDIAVEWESNGQPENNYKTTPPVLDSDGSFFLYSKLTVDKSRWQQGNVFSCSVMHEALHNHYTQKSLSLSPGK

SEQ ID NO: 5 - protein, 370 aa, Artificial
  Synthetic sequence
HKSDITLQEIIKTLNIVDQLKNYVNDLVPEFLPAPEDVETNCEWSAFSCFQKAQLKSANTGNNERIINVSIKKLKRKPPSTNAGRRQKHRLTCPSCDSYEKKPPKEFLERFKSLLQKMIHQHLSSRTHGSEDSGGGGSGGGGSDKTHTCPPCPAPEAAGGPSVFLFPPKPKDTLMISRTPEVTCVVVDVSHEDPEVKFNWYVDGVEVHNAKTKPREEQYNSTYRVVSVLTVLHQDWLNGKEYKCKVSNKALPAPIEKTISKAKGQPREPQVYTLPPSREEMTKNQVSLTCLVKGFYPSDIAVEWESNGQPENNYKTTPPVLDSDGSFFLYSKLTVDKSRWQQGNVFSCSVMHEALHNHYTQKSLSLSPGK

SEQ ID NO: 6 - protein, 370 aa, Artificial
  Synthetic sequence
HKSDITLQEIIKLIDIVDQLKNYVNDLVPEFLPAPEDVETNCEWSAFSCFQKAQLKSANTGNNERIINVSIKKLKRKPPSTNAGRRQKHRLTCPSCDSYEKKPPKEFLERFKSLLQKMIHQHLSSRTHGSEDSGGGGSGGGGSDKTHTCPPCPAPEAAGGPSVFLFPPKPKDTLMISRTPEVTCVVVDVSHEDPEVKFNWYVDGVEVHNAKTKPREEQYNSTYRVVSVLTVLHQDWLNGKEYKCKVSNKALPAPIEKTISKAKGQPREPQVYTLPPSREEMTKNQVSLTCLVKGFYPSDIAVEWESNGQPENNYKTTPPVLDSDGSFFLYSKLTVDKSRWQQGNVFSCSVMHEALHNHYTQKSLSLSPGK

SEQ ID NO: 7 - protein, 370 aa, Artificial
  Synthetic sequence
HKSDITLQEIIQLIDIVDQLKNYVNDLVPEFLPAPEDVETNCEWSAFSCFQKAQLKSANTGNNERIINVSIKKLKRKPPSTNAGRRQKHRLTCPSCDSYEKKPPKEFLERFKSLLQKMIHQHLSSRTHGSEDSGGGGSGGGGSDKTHTCPPCPAPEAAGGPSVFLFPPKPKDTLMISRTPEVTCVVVDVSHEDPEVKFNWYVDGVEVHNAKTKPREEQYNSTYRVVSVLTVLHQDWLNGKEYKCKVSNKALPAPIEKTISKAKGQPREPQVYTLPPSREEMTKNQVSLTCLVKGFYPSDIAVEWESNGQPENNYKTTPPVLDSDGSFFLYSKLTVDKSRWQQGNVFSCSVMHEALHNHYTQKSLSLSPGK

SEQ ID NO: 8 - protein, 372 aa, Artificial
  Synthetic sequence
HKSDITLQEIIMRQLIDIVDQLKNYVNDLVPEFLPAPEDVETNCEWSAFSCFQKAQLKSANTGNNERIINVSIKKLKRKPPSTNAGRRQKHRLTCPSCDSYEKKPPKEFLERFKSLLQKMIHQHLSSRTHGSEDSGGGGSGGGGSDKTHTCPPCPAPEAAGGPSVFLFPPKPKDTLMISRTPEVTCVVVDVSHEDPEVKFNWYVDGVEVHNAKTKPREEQYNSTYRVVSVLTVLHQDWLNGKEYKCKVSNKALPAPIEKTISKAKGQPREPQVYTLPPSREEMTKNQVSLTCLVKGFYPSDIAVEWESNGQPENNYKTTPPVLDSDGSFFLYSKLTVDKSRWQQGNVFSCSVMHEALHNHYTQKSLSLSPGK

SEQ ID NO: 9 - protein, 370 aa, Artificial
  Synthetic sequence
QGQNRTMIRMRQLIDIVDQLKNYVNDLVPEFLPAPEDVETNCEWSAFSCFQKAQLKSANTGNNERIINVSIKKLKRKPPSTNAGRRQKHRLTCPSCDSYEKKPPKEFLERFKSLLQKMIHQHLSSRTHGSEDSGGGGSGGGGSDKTHTCPPCPAPEAAGGPSVFLFPPKPKDTLMISRTPEVTCVVVDVSHEDPEVKFNWYVDGVEVHNAKTKPREEQYNSTYRVVSVLTVLHQDWLNGKEYKCKVSNKALPAPIEKTISKAKGQPREPQVYTLPPSREEMTKNQVSLTCLVKGFYPSDIAVEWESNGQPENNYKTTPPVLDSDGSFFLYSKLTVDKSRWQQGNVFSCSVMHEALHNHYTQKSLSLSPGK

SEQ ID NO: 10 - protein, 370 aa, Artificial
  Synthetic sequence
QGQDNHTIRMRQLIDIVDQLKNYVNDLVPEFLPAPEDVETNCEWSAFSCFQKAQLKSANTGNNERIINVSIKKLKRKPPSTNAGRRQKHRLTCPSCDSYEKKPPKEFLERFKSLLQKMIHQHLSSRTHGSEDSGGGGSGGGGSDKTHTCPPCPAPEAAGGPSVFLFPPKPKDTLMISRTPEVTCVVVDVSHEDPEVKFNWYVDGVEVHNAKTKPREEQYNSTYRVVSVLTVLHQDWLNGKEYKCKVSNKALPAPIEKTISKAKGQPREPQVYTLPPSREEMTKNQVSLTCLVKGFYPSDIAVEWESNGQPENNYKTTPPVLDSDGSFFLYSKLTVDKSRWQQGNVFSCSVMHEALHNHYTQKSLSLSPGK

SEQ ID NO: 11 - protein, 370 aa, Artificial
  Synthetic sequence
QGQDRHMIRMRQLINITDQLKNYVNDLVPEFLPAPEDVETNCEWSAFSCFQKAQLKSANTGNNERIINVSIKKLKRKPPSTNAGRRQKHRLTCPSCDSYEKKPPKEFLERFKSLLQKMIHQHLSSRTHGSEDSGGGGSGGGGSDKTHTCPPCPAPEAAGGPSVFLFPPKPKDTLMISRTPEVTCVVVDVSHEDPEVKFNWYVDGVEVHNAKTKPREEQYNSTYRVVSVLTVLHQDWLNGKEYKCKVSNKALPAPIEKTISKAKGQPREPQVYTLPPSREEMTKNQVSLTCLVKGFYPSDIAVEWESNGQPENNYKTTPPVLDSDGSFFLYSKLTVDKSRWQQGNVFSCSVMHEALHNHYTQKSLSLSPGK

SEQ ID NO: 12 - protein, 370 aa, Artificial
  Synthetic sequence
QGQDRHMIRMRQLIDIVDNLTNYVNDLVPEFLPAPEDVETNCEWSAFSCFQKAQLKSANTGNNERIINVSIKKLKRKPPSTNAGRRQKHRLTCPSCDSYEKKPPKEFLERFKSLLQKMIHQHLSSRTHGSEDSGGGGSGGGGSDKTHTCPPCPAPEAAGGPSVFLFPPKPKDTLMISRTPEVTCVVVDVSHEDPEVKFNWYVDGVEVHNAKTKPREEQYNSTYRVVSVLTVLHQDWLNGKEYKCKVSNKALPAPIEKTISKAKGQPREPQVYTLPPSREEMTKNQVSLTCLVKGFYPSDIAVEWESNGQPENNYKTTPPVLDSDGSFFLYSKLTVDKSRWQQGNVFSCSVMHEALHNHYTQKSLSLSPGK

SEQ ID NO: 13 - protein, 370 aa, Artificial
  Synthetic sequence
QGQDRHMIRMRQLIDIVDQLKNYVNDLVPEFLPAPEDVETNCEWSAFSCFQKAQLKSANTGNNERIINVSIKKLKNKTPSTNAGRRQKHRLTCPSCDSYEKKPPKEFLERFKSLLQKMIHQHLSSRTHGSEDSGGGGSGGGGSDKTHTCPPCPAPEAAGGPSVFLFPPKPKDTLMISRTPEVTCVVVDVSHEDPEVKFNWYVDGVEVHNAKTKPREEQYNSTYRVVSVLTVLHQDWLNGKEYKCKVSNKALPAPIEKTISKAKGQPREPQVYTLPPSREEMTKNQVSLTCLVKGFYPSDIAVEWESNGQPENNYKTTPPVLDSDGSFFLYSKLTVDKSRWQQGNVFSCSVMHEALHNHYTQKSLSLSPGK

SEQ ID NO: 14 - protein, 370 aa, Artificial
  Synthetic sequence
QGQDRHMIRMRQLIDIVDQLKNYVNDLVPEFLPAPEDVETNCEWSAFSCFQKAQLKSANTGNNERIINVSIKKLKRNSTSTNAGRRQKHRLTCPSCDSYEKKPPKEFLERFKSLLQKMIHQHLSSRTHGSEDSGGGGSGGGGSDKTHTCPPCPAPEAAGGPSVFLFPPKPKDTLMISRTPEVTCVVVDVSHEDPEVKFNWYVDGVEVHNAKTKPREEQYNSTYRVVSVLTVLHQDWLNGKEYKCKVSNKALPAPIEKTISKAKGQPREPQVYTLPPSREEMTKNQVSLTCLVKGFYPSDIAVEWESNGQPENNYKTTPPVLDSDGSFFLYSKLTVDKSRWQQGNVFSCSVMHEALHNHYTQKSLSLSPGK

SEQ ID NO: 15 - protein, 370 aa, Artificial
  Synthetic sequence
QGQDRHMIRMRQLIDIVDQLKNYVNDLVPEFLPAPEDVETNCEWSAFSCFQKAQLKSANTGNNERIINVSIKKLKRKPNSTNAGRRQKHRLTCPSCDSYEKKPPKEFLERFKSLLQKMIHQHLSSRTHGSEDSGGGGSGGGGSDKTHTCPPCPAPEAAGGPSVFLFPPKPKDTLMISRTPEVTCVVVDVSHEDPEVKFNWYVDGVEVHNAKTKPREEQYNSTYRVVSVLTVLHQDWLNGKEYKCKVSNKALPAPIEKTISKAKGQPREPQVYTLPPSREEMTKNQVSLTCLVKGFYPSDIAVEWESNGQPENNYKTTPPVLDSDGSFFLYSKLTVDKSRWQQGNVFSCSVMHEALHNHYTQKSLSLSPGK

SEQ ID NO: 16 - protein, 370 aa, Artificial
  Synthetic sequence
QGQDRHMIRMRQLIDIVDQLKNYVNDLVPEFLPAPEDVETNCEWSAFSCFQKAQLKSANTGNNERIINVSIKKLKRKPPNTTAGRRQKHRLTCPSCDSYEKKPPKEFLERFKSLLQKMIHQHLSSRTHGSEDSGGGGSGGGGSDKTHTCPPCPAPEAAGGPSVFLFPPKPKDTLMISRTPEVTCVVVDVSHEDPEVKFNWYVDGVEVHNAKTKPREEQYNSTYRVVSVLTVLHQDWLNGKEYKCKVSNKALPAPIEKTISKAKGQPREPQVYTLPPSREEMTKNQVSLTCLVKGFYPSDIAVEWESNGQPENNYKTTPPVLDSDGSFFLYSKLTVDKSRWQQGNVFSCSVMHEALHNHYTQKSLSLSPGK

SEQ ID NO: 17 - protein, 370 aa, Artificial
  Synthetic sequence
QGQDRHMIRMRQLIDIVDQLKNYVNDLVPEFLPAPEDVETNCEWSAFSCFQKAQLKSANTGNNERIINVSIKKLKRKPPSTNATRRQKHRLTCPSCDSYEKKPPKEFLERFKSLLQKMIHQHLSSRTHGSEDSGGGGSGGGGSDKTHTCPPCPAPEAAGGPSVFLFPPKPKDTLMISRTPEVTCVVVDVSHEDPEVKFNWYVDGVEVHNAKTKPREEQYNSTYRVVSVLTVLHQDWLNGKEYKCKVSNKALPAPIEKTISKAKGQPREPQVYTLPPSREEMTKNQVSLTCLVKGFYPSDIAVEWESNGQPENNYKTTPPVLDSDGSFFLYSKLTVDKSRWQQGNVFSCSVMHEALHNHYTQKSLSLSPGK

SEQ ID NO: 18 - protein, 370 aa, Artificial
  Synthetic sequence
QGQDRHMIRMRQLIDIVDQLKNYVNDLVPEFLPAPEDVETNCEWSAFSCFQKAQLKSANTGNNERIINVSIKKLKRKPPSTNAGRRQKHRLTCPSCDSYEKKPPKEFLERFKSLLQKMINQTLSSRTHGSEDSGGGGSGGGGSDKTHTCPPCPAPEAAGGPSVFLFPPKPKDTLMISRTPEVTCVVVDVSHEDPEVKFNWYVDGVEVHNAKTKPREEQYNSTYRVVSVLTVLHQDWLNGKEYKCKVSNKALPAPIEKTISKAKGQPREPQVYTLPPSREEMTKNQVSLTCLVKGFYPSDIAVEWESNGQPENNYKTTPPVLDSDGSFFLYSKLTVDKSRWQQGNVFSCSVMHEALHNHYTQKSLSLSPGK

SEQ ID NO: 19 - protein, 370 aa, Artificial
  Synthetic sequence
QGQDRHMIRMRQLIDIVDQLKNYVNDLVPEFLPAPENVTTNCEWSAFSCFQKAQLKSANTGNNERIINVSIKKLKRKPPSTNAGRRQKHRLTCPSCDSYEKKPPKEFLERFKSLLQKMIHQHLSSRTHGSEDSGGGGSGGGGSDKTHTCPPCPAPEAAGGPSVFLFPPKPKDTLMISRTPEVTCVVVDVSHEDPEVKFNWYVDGVEVHNAKTKPREEQYNSTYRVVSVLTVLHQDWLNGKEYKCKVSNKALPAPIEKTISKAKGQPREPQVYTLPPSREEMTKNQVSLTCLVKGFYPSDIAVEWESNGQPENNYKTTPPVLDSDGSFFLYSKLTVDKSRWQQGNVFSCSVMHEALHNHYTQKSLSLSPGK

SEQ ID NO: 20 - protein, 370 aa, Artificial
  Synthetic sequence
QGQDRHMIRMRQLIDIVDQLKNYVNDLVPEFLPAPEDVETNCEWSAFSCFQKAQLKSANTGNNERIINVSIEKLKRKPPSTNAGRRQKHRLTCPSCDSYEKKPPKEFLERFKSLLQKMIHQHLSSRTHGSEDSGGGGSGGGGSDKTHTCPPCPAPEAAGGPSVFLFPPKPKDTLMISRTPEVTCVVVDVSHEDPEVKFNWYVDGVEVHNAKTKPREEQYNSTYRVVSVLTVLHQDWLNGKEYKCKVSNKALPAPIEKTISKAKGQPREPQVYTLPPSREEMTKNQVSLTCLVKGFYPSDIAVEWESNGQPENNYKTTPPVLDSDGSFFLYSKLTVDKSRWQQGNVFSCSVMHEALHNHYTQKSLSLSPGK

SEQ ID NO: 21 - protein, 370 aa, Artificial
  Synthetic sequence
QGQDRHMQRMRQLIDIVDQLKNYVNDLVPEFLPAPEDVETNCEWSAFSCFQKAQLKSANTGNNERIINVSIKKLKRKPESTNAGRRQKHRLTCPSCDSYEKKPPKEFLERFKSLLQKMIHQHLSSRTHGSEDSGGGGSGGGGSDKTHTCPPCPAPEAAGGPSVFLFPPKPKDTLMISRTPEVTCVVVDVSHEDPEVKFNWYVDGVEVHNAKTKPREEQYNSTYRVVSVLTVLHQDWLNGKEYKCKVSNKALPAPIEKTISKAKGQPREPQVYTLPPSREEMTKNQVSLTCLVKGFYPSDIAVEWESNGQPENNYKTTPPVLDSDGSFFLYSKLTVDKSRWQQGNVFSCSVMHEALHNHYTQKSLSLSPGK

SEQ ID NO: 22 - protein, 370 aa, Artificial
  Synthetic sequence
QGQDRHMIRMRQLIDIVDQLKNYVNDLVPEFLPAPEDVETNCEWSAFSCFQKAQLKSANTGNNERIINVSIKKLKRDAPSTNAGRRQKHRLTCPSCDSYEKKPPKEFLERFKSLLQKMIHQHLSSRTHGSEDSGGGGSGGGGSDKTHTCPPCPAPEAAGGPSVFLFPPKPKDTLMISRTPEVTCVVVDVSHEDPEVKFNWYVDGVEVHNAKTKPREEQYNSTYRVVSVLTVLHQDWLNGKEYKCKVSNKALPAPIEKTISKAKGQPREPQVYTLPPSREEMTKNQVSLTCLVKGFYPSDIAVEWESNGQPENNYKTTPPVLDSDGSFFLYSKLTVDKSRWQQGNVFSCSVMHEALHNHYTQKSLSLSPGK

SEQ ID NO: 23 - protein, 367 aa, Artificial
  Synthetic sequence
QGQDRHMIRMRQLIDIVDQLKNYVNDLVPEFLPAPEDVETNCEWSAFSCFQKAQLKSANTGNNERIINVSIKKLKRKPPSTNAGKHRLTCPSCDSYEKKPPKEFLERFKSLLQKMIHQHLSSRTHGSEDSGGGGSGGGGSDKTHTCPPCPAPEAAGGPSVFLFPPKPKDTLMISRTPEVTCVVVDVSHEDPEVKFNWYVDGVEVHNAKTKPREEQYNSTYRVVSVLTVLHQDWLNGKEYKCKVSNKALPAPIEKTISKAKGQPREPQVYTLPPSREEMTKNQVSLTCLVKGFYPSDIAVEWESNGQPENNYKTTPPVLDSDGSFFLYSKLTVDKSRWQQGNVFSCSVMHEALHNHYTQKSLSLSPGK

SEQ ID NO: 24 - protein, 368 aa, Artificial
  Synthetic sequence
QGQDRHMIRMRQLIDIVDQLKNYVNDLVPEFLPAPEDVETNCEWSAFSCFQKAQLKSANTGNNERIINVSIKKLKRKSTNAGRRQKHRLTCPSCDSYEKKPPKEFLERFKSLLQKMIHQHLSSRTHGSEDSGGGGSGGGGSDKTHTCPPCPAPEAAGGPSVFLFPPKPKDTLMISRTPEVTCVVVDVSHEDPEVKFNWYVDGVEVHNAKTKPREEQYNSTYRVVSVLTVLHQDWLNGKEYKCKVSNKALPAPIEKTISKAKGQPREPQVYTLPPSREEMTKNQVSLTCLVKGFYPSDIAVEWESNGQPENNYKTTPPVLDSDGSFFLYSKLTVDKSRWQQGNVFSCSVMHEALHNHYTQKSLSLSPGK

SEQ ID NO: 25 - protein, 361 aa, Artificial
  Synthetic sequence
MRQLIDIVDQLKNYVNDLVPEFLPAPEDVETNCEWSAFSCFQKAQLKSANTGNNERIINVSIKKLKRKPPSTNAGRRQKHRLTCPSCDSYEKKPPKEFLERFKSLLQKMIHQHLSSRTHGSEDSGGGGSGGGGSDKTHTCPPCPAPEAAGGPSVFLFPPKPKDTLMISRTPEVTCVVVDVSHEDPEVKFNWYVDGVEVHNAKTKPREEQYNSTYRVVSVLTVLHQDWLNGKEYKCKVSNKALPAPIEKTISKAKGQPREPQVYTLPPSREEMTKNQVSLTCLVKGFYPSDIAVEWESNGQPENNYKTTPPVLDSDGSFFLYSKLTVDKSRWQQGNVFSCSVMHEALHNHYTQKSLSLSPGK

SEQ ID NO: 26 - protein, 359 aa, Artificial
  Synthetic sequence
MRQLIDIVDQLKNYVNDLVPEFLPAPEDVETNCEWSAFSCFQKAQLKSANTGNNERIINVSIKKLKRKSTNAGRRQKHRLTCPSCDSYEKKPPKEFLERFKSLLQKMIHQHLSSRTHGSEDSGGGGSGGGGSDKTHTCPPCPAPEAAGGPSVFLFPPKPKDTLMISRTPEVTCVVVDVSHEDPEVKFNWYVDGVEVHNAKTKPREEQYNSTYRVVSVLTVLHQDWLNGKEYKCKVSNKALPAPIEKTISKAKGQPREPQVYTLPPSREEMTKNQVSLTCLVKGFYPSDIAVEWESNGQPENNYKTTPPVLDSDGSFFLYSKLTVDKSRWQQGNVFSCSVMHEALHNHYTQKSLSLSPGK

SEQ ID NO: 27 - protein, 361 aa, Artificial
  Synthetic sequence
MRQLIDIVDNLTNYVNDLVPEFLPAPEDVETNCEWSAFSCFQKAQLKSANTGNNERIINVSIKKLKRKPPSTNAGRRQKHRLTCPSCDSYEKKPPKEFLERFKSLLQKMIHQHLSSRTHGSEDSGGGGSGGGGSDKTHTCPPCPAPEAAGGPSVFLFPPKPKDTLMISRTPEVTCVVVDVSHEDPEVKFNWYVDGVEVHNAKTKPREEQYNSTYRVVSVLTVLHQDWLNGKEYKCKVSNKALPAPIEKTISKAKGQPREPQVYTLPPSREEMTKNQVSLTCLVKGFYPSDIAVEWESNGQPENNYKTTPPVLDSDGSFFLYSKLTVDKSRWQQGNVFSCSVMHEALHNHYTQKSLSLSPGK

SEQ ID NO: 28 - protein, 362 aa, Artificial
  Synthetic sequence
QGQDRHMIRMRQLIDIVDNLTNYVNDLVPEFLPAPEDVETNAEWSAFSCFQKAQLKSANTGNNERIINVSIKKLKRKPPSTNATTPSCDSYEKKPPKEFLERFKSLLQKMIHQHLSSRTHGSEDSGGGGSGGGGSDKTHTCPPCPAPEAAGGPSVFLFPPKPKDTLMISRTPEVTCVVVDVSHEDPEVKFNWYVDGVEVHNAKTKPREEQYNSTYRVVSVLTVLHQDWLNGKEYKCKVSNKALPAPIEKTISKAKGQPREPQVYTLPPSREEMTKNQVSLTCLVKGFYPSDIAVEWESNGQPENNYKTTPPVLDSDGSFFLYSKLTVDKSRWQQGNVFSCSVMHEALHNHYTQKSLSLSPGK

SEQ ID NO: 29 - protein, 368 aa, Artificial
  Synthetic sequence
HKSDITLQEMRQLIDIVDQLKNYVNDLVPEFLPAPEDVETNCEWSAFSCFQKAQLKSANTGNNERIINVSIKKLKRKSTNAGRRQKHRLTCPSCDSYEKKPPKEFLERFKSLLQKMIHQHLSSRTHGSEDSGGGGSGGGGSDKTHTCPPCPAPEAAGGPSVFLFPPKPKDTLMISRTPEVTCVVVDVSHEDPEVKFNWYVDGVEVHNAKTKPREEQYNSTYRVVSVLTVLHQDWLNGKEYKCKVSNKALPAPIEKTISKAKGQPREPQVYTLPPSREEMTKNQVSLTCLVKGFYPSDIAVEWESNGQPENNYKTTPPVLDSDGSFFLYSKLTVDKSRWQQGNVFSCSVMHEALHNHYTQKSLSLSPGK

SEQ ID NO: 30 - protein, 370 aa, Artificial
  Synthetic sequence
HKSDITLQEMRQLIDIVDQLKNYVNDLVPEFLPAPEDVETNCEWSAFSCFQKAQLKSANTGNNERIINVSIKKLKRKPPSTNAGRRQKHRLTCPSCDSYEKKPPKEFLERFKSLLQNMTHQHLSSRTHGSEDSGGGGSGGGGSDKTHTCPPCPAPEAAGGPSVFLFPPKPKDTLMISRTPEVTCVVVDVSHEDPEVKFNWYVDGVEVHNAKTKPREEQYNSTYRVVSVLTVLHQDWLNGKEYKCKVSNKALPAPIEKTISKAKGQPREPQVYTLPPSREEMTKNQVSLTCLVKGFYPSDIAVEWESNGQPENNYKTTPPVLDSDGSFFLYSKLTVDKSRWQQGNVFSCSVMHEALHNHYTQKSLSLSPGK

SEQ ID NO: 31 - protein, 370 aa, Artificial
  Synthetic sequence
HKSDITLQEMRQLIDIVDQLKNYVNDLVPEFLPAPENVTTNCEWSAFSCFQKAQLKSANTGNNERIINVSIKKLKRKPPSTNAGRRQKHRLTCPSCDSYEKKPPKEFLERFKSLLQKMIHQHLSSRTHGSEDSGGGGSGGGGSDKTHTCPPCPAPEAAGGPSVFLFPPKPKDTLMISRTPEVTCVVVDVSHEDPEVKFNWYVDGVEVHNAKTKPREEQYNSTYRVVSVLTVLHQDWLNGKEYKCKVSNKALPAPIEKTISKAKGQPREPQVYTLPPSREEMTKNQVSLTCLVKGFYPSDIAVEWESNGQPENNYKTTPPVLDSDGSFFLYSKLTVDKSRWQQGNVFSCSVMHEALHNHYTQKSLSLSPGK

SEQ ID NO: 32 - protein, 370 aa, Artificial
  Synthetic sequence
HKSDITLQEMRQLINITDQLKNYVNDLVPEFLPAPEDVETNCEWSAFSCFQKAQLKSANTGNNERIINVSIKKLKRKPPSTNAGRRQKHRLTCPSCDSYEKKPPKEFLERFKSLLQKMIHQHLSSRTHGSEDSGGGGSGGGGSDKTHTCPPCPAPEAAGGPSVFLFPPKPKDTLMISRTPEVTCVVVDVSHEDPEVKFNWYVDGVEVHNAKTKPREEQYNSTYRVVSVLTVLHQDWLNGKEYKCKVSNKALPAPIEKTISKAKGQPREPQVYTLPPSREEMTKNQVSLTCLVKGFYPSDIAVEWESNGQPENNYKTTPPVLDSDGSFFLYSKLTVDKSRWQQGNVFSCSVMHEALHNHYTQKSLSLSPGK

SEQ ID NO: 33 - protein, 450 aa, Artificial
  Synthetic sequence
QVQLVQSGAEVKKPGSSVKVSCKASGGTFSSYAISWVRQAPGQGLEWMGLIIPMFDTAGYAQKFQGRVAITVDESTSTAYMELSSLRSEDTAVYYCARAEHSSTGTFDYWGQGTLVTVSSASTKGPSVFPLAPSSKSTSGGTAALGCLVKDYFPEPVTVSWNSGALTSGVHTFPAVLQSSGLYSLSSVVTVPSSSLGTQTYICNVNHKPSNTKVDKKVEPKSCDKTHTCPPCPAPEAAGGPSVFLFPPKPKDTLMISRTPEVTCVVVDVSHEDPEVKFNWYVDGVEVHNAKTKPREEQYNSTYRVVSVLTVLHQDWLNGKEYKCKVSNKALPAPIEKTISKAKGQPREPQVCTLPPSRDELTKNQVSLSCAVKGFYPSDIAVEWESNGQPENNYKTTPPVLDSDGSFFLVSKLTVDKSRWQQGNVFSCSVMHEALHNHYTQKSLSLSPGK

SEQ ID NO: 34 - protein, 214 aa, Artificial
  Synthetic sequence
DIQMTQSPSSVSASVGDRVTITCRASQGISSWLAWYQQKPGKAPKLLISAASSLQSGVPSRFSGSGSGTDFTLTISSLQPEDFATYYCQQANHLPFTFGGGTKVEIKRTVAAPSVFIFPPSDEQLKSGTASVVCLLNNFYPREAKVQWKVDNALQSGNSQESVTEQDSKDSTYSLSSTLTLSKADYEKHKVYACEVTHQGLSSPVTKSFNRGEC

SEQ ID NO: 35 - protein, 582 aa, Artificial
  Synthetic sequence
QVQLVQSGAEVKKPGSSVKVSCKASGGTFSSYAISWVRQAPGQGLEWMGLIIPMFDTAGYAQKFQGRVAITVDESTSTAYMELSSLRSEDTAVYYCARAEHSSTGTFDYWGQGTLVTVSSASTKGPSVFPLAPSSKSTSGGTAALGCLVKDYFPEPVTVSWNSGALTSGVHTFPAVLQSSGLYSLSSVVTVPSSSLGTQTYICNVNHKPSNTKVDKKVEPKSCDKTHTCPPCPAPEAAGGPSVFLFPPKPKDTLMISRTPEVTCVVVDVSHEDPEVKFNWYVDGVEVHNAKTKPREEQYNSTYRVVSVLTVLHQDWLNGKEYKCKVSNKALPAPIEKTISKAKGQPREPQVYTLPPSREEMTKNQVSLTCLVKGFYPSDIAVEWESNGQPENNYKTTPPVLDSDGSFFLYSKLTVDKSRWQQGNVFSCSVMHEALHNHYTQKSLSLSPGQGQDRHMIRMRQLIDIVDQLKNYVNDLVPEFLPAPEDVETNCEWSAFSCFQKAQLKSANTGNNERIINVSIKKLKRKPPSTNAGRRQKHRLTCPSCDSYEKKPPKEFLERFKSLLQKMIHQHLSSRTHGSEDS

SEQ ID NO: 36 - protein, 582 aa, Artificial
  Synthetic sequence
QVQLVQSGAEVKKPGSSVKVSCKASGGTFSSYAISWVRQAPGQGLEWMGLIIPMFDTAGYAQKFQGRVAITVDESTSTAYMELSSLRSEDTAVYYCARAEHSSTGTFDYWGQGTLVTVSSASTKGPSVFPLAPSSKSTSGGTAALGCLVKDYFPEPVTVSWNSGALTSGVHTFPAVLQSSGLYSLSSVVTVPSSSLGTQTYICNVNHKPSNTKVDKKVEPKSCDKTHTCPPCPAPEAAGGPSVFLFPPKPKDTLMISRTPEVTCVVVDVSHEDPEVKFNWYVDGVEVHNAKTKPREEQYNSTYRVVSVLTVLHQDWLNGKEYKCKVSNKALPAPIEKTISKAKGQPREPQVYTLPPSREEMTKNQVSLTCLVKGFYPSDIAVEWESNGQPENNYKTTPPVLDSDGSFFLYSKLTVDKSRWQQGNVFSCSVMHEALHNHYTQKSLSLSPGHKSDIHMIRMRQLIDIVDQLKNYVNDLVPEFLPAPEDVETNCEWSAFSCFQKAQLKSANTGNNERIINVSIKKLKRKPPSTNAGRRQKHRLTCPSCDSYEKKPPKEFLERFKSLLQKMIHQHLSSRTHGSEDS

SEQ ID NO: 37 - protein, 582 aa, Artificial
  Synthetic sequence
QVQLVQSGAEVKKPGSSVKVSCKASGGTFSSYAISWVRQAPGQGLEWMGLIIPMFDTAGYAQKFQGRVAITVDESTSTAYMELSSLRSEDTAVYYCARAEHSSTGTFDYWGQGTLVTVSSASTKGPSVFPLAPSSKSTSGGTAALGCLVKDYFPEPVTVSWNSGALTSGVHTFPAVLQSSGLYSLSSVVTVPSSSLGTQTYICNVNHKPSNTKVDKKVEPKSCDKTHTCPPCPAPEAAGGPSVFLFPPKPKDTLMISRTPEVTCVVVDVSHEDPEVKFNWYVDGVEVHNAKTKPREEQYNSTYRVVSVLTVLHQDWLNGKEYKCKVSNKALPAPIEKTISKAKGQPREPQVYTLPPSREEMTKNQVSLTCLVKGFYPSDIAVEWESNGQPENNYKTTPPVLDSDGSFFLYSKLTVDKSRWQQGNVFSCSVMHEALHNHYTQKSLSLSPGHKCDIHMIRMRQLIDIVDQLKNYVNDLVPEFLPAPEDVETNCEWSAFSCFQKAQLKSANTGNNERIINVSIKKLKRKPPSTNAGRRQKHRLTCPSCDSYEKKPPKEFLERFKSLLQKMIHQHCSSRTHGSEDS

SEQ ID NO: 38 - protein, 582 aa, Artificial
  Synthetic sequence
QVQLVQSGAEVKKPGSSVKVSCKASGGTFSSYAISWVRQAPGQGLEWMGLIIPMFDTAGYAQKFQGRVAITVDESTSTAYMELSSLRSEDTAVYYCARAEHSSTGTFDYWGQGTLVTVSSASTKGPSVFPLAPSSKSTSGGTAALGCLVKDYFPEPVTVSWNSGALTSGVHTFPAVLQSSGLYSLSSVVTVPSSSLGTQTYICNVNHKPSNTKVDKKVEPKSCDKTHTCPPCPAPEAAGGPSVFLFPPKPKDTLMISRTPEVTCVVVDVSHEDPEVKFNWYVDGVEVHNAKTKPREEQYNSTYRVVSVLTVLHQDWLNGKEYKCKVSNKALPAPIEKTISKAKGQPREPQVYTLPPSREEMTKNQVSLTCLVKGFYPSDIAVEWESNGQPENNYKTTPPVLDSDGSFFLYSKLTVDKSRWQQGNVFSCSVMHEALHNHYTQKSLSLSPGQGQNRTMIRMRQLIDIVDQLKNYVNDLVPEFLPAPEDVETNCEWSAFSCFQKAQLKSANTGNNERIINVSIKKLKRKPPSTNAGRRQKHRLTCPSCDSYEKKPPKEFLERFKSLLQKMIHQHLSSRTHGSEDS

SEQ ID NO: 39 - protein, 582 aa, Artificial
  Synthetic sequence
QVQLVQSGAEVKKPGSSVKVSCKASGGTFSSYAISWVRQAPGQGLEWMGLIIPMFDTAGYAQKFQGRVAITVDESTSTAYMELSSLRSEDTAVYYCARAEHSSTGTFDYWGQGTLVTVSSASTKGPSVFPLAPSSKSTSGGTAALGCLVKDYFPEPVTVSWNSGALTSGVHTFPAVLQSSGLYSLSSVVTVPSSSLGTQTYICNVNHKPSNTKVDKKVEPKSCDKTHTCPPCPAPEAAGGPSVFLFPPKPKDTLMISRTPEVTCVVVDVSHEDPEVKFNWYVDGVEVHNAKTKPREEQYNSTYRVVSVLTVLHQDWLNGKEYKCKVSNKALPAPIEKTISKAKGQPREPQVYTLPPSREEMTKNQVSLTCLVKGFYPSDIAVEWESNGQPENNYKTTPPVLDSDGSFFLYSKLTVDKSRWQQGNVFSCSVMHEALHNHYTQKSLSLSPGQGQDNHTIRMRQLIDIVDQLKNYVNDLVPEFLPAPEDVETNCEWSAFSCFQKAQLKSANTGNNERIINVSIKKLKRKPPSTNAGRRQKHRLTCPSCDSYEKKPPKEFLERFKSLLQKMIHQHLSSRTHGSEDS

SEQ ID NO: 40 - protein, 582 aa, Artificial
  Synthetic sequence
QVQLVQSGAEVKKPGSSVKVSCKASGGTFSSYAISWVRQAPGQGLEWMGLIIPMFDTAGYAQKFQGRVAITVDESTSTAYMELSSLRSEDTAVYYCARAEHSSTGTFDYWGQGTLVTVSSASTKGPSVFPLAPSSKSTSGGTAALGCLVKDYFPEPVTVSWNSGALTSGVHTFPAVLQSSGLYSLSSVVTVPSSSLGTQTYICNVNHKPSNTKVDKKVEPKSCDKTHTCPPCPAPEAAGGPSVFLFPPKPKDTLMISRTPEVTCVVVDVSHEDPEVKFNWYVDGVEVHNAKTKPREEQYNSTYRVVSVLTVLHQDWLNGKEYKCKVSNKALPAPIEKTISKAKGQPREPQVYTLPPSREEMTKNQVSLTCLVKGFYPSDIAVEWESNGQPENNYKTTPPVLDSDGSFFLYSKLTVDKSRWQQGNVFSCSVMHEALHNHYTQKSLSLSPGQGQDRHMIRMRQLINITDQLKNYVNDLVPEFLPAPEDVETNCEWSAFSCFQKAQLKSANTGNNERIINVSIKKLKRKPPSTNAGRRQKHRLTCPSCDSYEKKPPKEFLERFKSLLQKMIHQHLSSRTHGSEDS

SEQ ID NO: 41 - protein, 582 aa, Artificial
  Synthetic sequence
QVQLVQSGAEVKKPGSSVKVSCKASGGTFSSYAISWVRQAPGQGLEWMGLIIPMFDTAGYAQKFQGRVAITVDESTSTAYMELSSLRSEDTAVYYCARAEHSSTGTFDYWGQGTLVTVSSASTKGPSVFPLAPSSKSTSGGTAALGCLVKDYFPEPVTVSWNSGALTSGVHTFPAVLQSSGLYSLSSVVTVPSSSLGTQTYICNVNHKPSNTKVDKKVEPKSCDKTHTCPPCPAPEAAGGPSVFLFPPKPKDTLMISRTPEVTCVVVDVSHEDPEVKFNWYVDGVEVHNAKTKPREEQYNSTYRVVSVLTVLHQDWLNGKEYKCKVSNKALPAPIEKTISKAKGQPREPQVYTLPPSREEMTKNQVSLTCLVKGFYPSDIAVEWESNGQPENNYKTTPPVLDSDGSFFLYSKLTVDKSRWQQGNVFSCSVMHEALHNHYTQKSLSLSPGQGQDRHMIRMRQLIDIVDNLTNYVNDLVPEFLPAPEDVETNCEWSAFSCFQKAQLKSANTGNNERIINVSIKKLKRKPPSTNAGRRQKHRLTCPSCDSYEKKPPKEFLERFKSLLQKMIHQHLSSRTHGSEDS

SEQ ID NO: 42 - protein, 582 aa, Artificial
  Synthetic sequence
QVQLVQSGAEVKKPGSSVKVSCKASGGTFSSYAISWVRQAPGQGLEWMGLIIPMFDTAGYAQKFQGRVAITVDESTSTAYMELSSLRSEDTAVYYCARAEHSSTGTFDYWGQGTLVTVSSASTKGPSVFPLAPSSKSTSGGTAALGCLVKDYFPEPVTVSWNSGALTSGVHTFPAVLQSSGLYSLSSVVTVPSSSLGTQTYICNVNHKPSNTKVDKKVEPKSCDKTHTCPPCPAPEAAGGPSVFLFPPKPKDTLMISRTPEVTCVVVDVSHEDPEVKFNWYVDGVEVHNAKTKPREEQYNSTYRVVSVLTVLHQDWLNGKEYKCKVSNKALPAPIEKTISKAKGQPREPQVYTLPPSREEMTKNQVSLTCLVKGFYPSDIAVEWESNGQPENNYKTTPPVLDSDGSFFLYSKLTVDKSRWQQGNVFSCSVMHEALHNHYTQKSLSLSPGQGQDRHMIRMRQLIDIVDQLKNYVNDLVPEFLPAPEDVETNCEWSAFSCFQKAQLKSANTGNNERIINVSIKKLKNKTPSTNAGRRQKHRLTCPSCDSYEKKPPKEFLERFKSLLQKMIHQHLSSRTHGSEDS

SEQ ID NO: 43 - protein, 582 aa, Artificial
  Synthetic sequence
QVQLVQSGAEVKKPGSSVKVSCKASGGTFSSYAISWVRQAPGQGLEWMGLIIPMFDTAGYAQKFQGRVAITVDESTSTAYMELSSLRSEDTAVYYCARAEHSSTGTFDYWGQGTLVTVSSASTKGPSVFPLAPSSKSTSGGTAALGCLVKDYFPEPVTVSWNSGALTSGVHTFPAVLQSSGLYSLSSVVTVPSSSLGTQTYICNVNHKPSNTKVDKKVEPKSCDKTHTCPPCPAPEAAGGPSVFLFPPKPKDTLMISRTPEVTCVVVDVSHEDPEVKFNWYVDGVEVHNAKTKPREEQYNSTYRVVSVLTVLHQDWLNGKEYKCKVSNKALPAPIEKTISKAKGQPREPQVYTLPPSREEMTKNQVSLTCLVKGFYPSDIAVEWESNGQPENNYKTTPPVLDSDGSFFLYSKLTVDKSRWQQGNVFSCSVMHEALHNHYTQKSLSLSPGQGQDRHMIRMRQLIDIVDQLKNYVNDLVPEFLPAPEDVETNCEWSAFSCFQKAQLKSANTGNNERIINVSIKKLKRNSTSTNAGRRQKHRLTCPSCDSYEKKPPKEFLERFKSLLQKMIHQHLSSRTHGSEDS

SEQ ID NO: 44 - protein, 582 aa, Artificial
  Synthetic sequence
QVQLVQSGAEVKKPGSSVKVSCKASGGTFSSYAISWVRQAPGQGLEWMGLIIPMFDTAGYAQKFQGRVAITVDESTSTAYMELSSLRSEDTAVYYCARAEHSSTGTFDYWGQGTLVTVSSASTKGPSVFPLAPSSKSTSGGTAALGCLVKDYFPEPVTVSWNSGALTSGVHTFPAVLQSSGLYSLSSVVTVPSSSLGTQTYICNVNHKPSNTKVDKKVEPKSCDKTHTCPPCPAPEAAGGPSVFLFPPKPKDTLMISRTPEVTCVVVDVSHEDPEVKFNWYVDGVEVHNAKTKPREEQYNSTYRVVSVLTVLHQDWLNGKEYKCKVSNKALPAPIEKTISKAKGQPREPQVYTLPPSREEMTKNQVSLTCLVKGFYPSDIAVEWESNGQPENNYKTTPPVLDSDGSFFLYSKLTVDKSRWQQGNVFSCSVMHEALHNHYTQKSLSLSPGQGQDRHMIRMRQLIDIVDQLKNYVNDLVPEFLPAPEDVETNCEWSAFSCFQKAQLKSANTGNNERIINVSIKKLKRKPNSTNAGRRQKHRLTCPSCDSYEKKPPKEFLERFKSLLQKMIHQHLSSRTHGSEDS

SEQ ID NO: 45 - protein, 582 aa, Artificial
  Synthetic sequence
QVQLVQSGAEVKKPGSSVKVSCKASGGTFSSYAISWVRQAPGQGLEWMGLIIPMFDTAGYAQKFQGRVAITVDESTSTAYMELSSLRSEDTAVYYCARAEHSSTGTFDYWGQGTLVTVSSASTKGPSVFPLAPSSKSTSGGTAALGCLVKDYFPEPVTVSWNSGALTSGVHTFPAVLQSSGLYSLSSVVTVPSSSLGTQTYICNVNHKPSNTKVDKKVEPKSCDKTHTCPPCPAPEAAGGPSVFLFPPKPKDTLMISRTPEVTCVVVDVSHEDPEVKFNWYVDGVEVHNAKTKPREEQYNSTYRVVSVLTVLHQDWLNGKEYKCKVSNKALPAPIEKTISKAKGQPREPQVYTLPPSREEMTKNQVSLTCLVKGFYPSDIAVEWESNGQPENNYKTTPPVLDSDGSFFLYSKLTVDKSRWQQGNVFSCSVMHEALHNHYTQKSLSLSPGQGQDRHMIRMRQLIDIVDQLKNYVNDLVPEFLPAPEDVETNCEWSAFSCFQKAQLKSANTGNNERIINVSIKKLKRKPPNTTAGRRQKHRLTCPSCDSYEKKPPKEFLERFKSLLQKMIHQHLSSRTHGSEDS

SEQ ID NO: 46 - protein, 582 aa, Artificial
  Synthetic sequence
QVQLVQSGAEVKKPGSSVKVSCKASGGTFSSYAISWVRQAPGQGLEWMGLIIPMFDTAGYAQKFQGRVAITVDESTSTAYMELSSLRSEDTAVYYCARAEHSSTGTFDYWGQGTLVTVSSASTKGPSVFPLAPSSKSTSGGTAALGCLVKDYFPEPVTVSWNSGALTSGVHTFPAVLQSSGLYSLSSVVTVPSSSLGTQTYICNVNHKPSNTKVDKKVEPKSCDKTHTCPPCPAPEAAGGPSVFLFPPKPKDTLMISRTPEVTCVVVDVSHEDPEVKFNWYVDGVEVHNAKTKPREEQYNSTYRVVSVLTVLHQDWLNGKEYKCKVSNKALPAPIEKTISKAKGQPREPQVYTLPPSREEMTKNQVSLTCLVKGFYPSDIAVEWESNGQPENNYKTTPPVLDSDGSFFLYSKLTVDKSRWQQGNVFSCSVMHEALHNHYTQKSLSLSPGQGQDRHMIRMRQLIDIVDQLKNYVNDLVPEFLPAPEDVETNCEWSAFSCFQKAQLKSANTGNNERIINVSIKKLKRKPPSTNATRRQKHRLTCPSCDSYEKKPPKEFLERFKSLLQKMIHQHLSSRTHGSEDS

SEQ ID NO: 47 - protein, 582 aa, Artificial
  Synthetic sequence
QVQLVQSGAEVKKPGSSVKVSCKASGGTFSSYAISWVRQAPGQGLEWMGLIIPMFDTAGYAQKFQGRVAITVDESTSTAYMELSSLRSEDTAVYYCARAEHSSTGTFDYWGQGTLVTVSSASTKGPSVFPLAPSSKSTSGGTAALGCLVKDYFPEPVTVSWNSGALTSGVHTFPAVLQSSGLYSLSSVVTVPSSSLGTQTYICNVNHKPSNTKVDKKVEPKSCDKTHTCPPCPAPEAAGGPSVFLFPPKPKDTLMISRTPEVTCVVVDVSHEDPEVKFNWYVDGVEVHNAKTKPREEQYNSTYRVVSVLTVLHQDWLNGKEYKCKVSNKALPAPIEKTISKAKGQPREPQVYTLPPSREEMTKNQVSLTCLVKGFYPSDIAVEWESNGQPENNYKTTPPVLDSDGSFFLYSKLTVDKSRWQQGNVFSCSVMHEALHNHYTQKSLSLSPGQGQDRHMIRMRQLIDIVDQLKNYVNDLVPEFLPAPEDVETNCEWSAFSCFQKAQLKSANTGNNERIINVSIKKLKRKPPSTNAGRRQKHRLTCPSCDSYEKKPPKEFLERFKSLLQKMINQTLSSRTHGSEDS

SEQ ID NO: 48 - protein, 582 aa, Artificial
  Synthetic sequence
QVQLVQSGAEVKKPGSSVKVSCKASGGTFSSYAISWVRQAPGQGLEWMGLIIPMFDTAGYAQKFQGRVAITVDESTSTAYMELSSLRSEDTAVYYCARAEHSSTGTFDYWGQGTLVTVSSASTKGPSVFPLAPSSKSTSGGTAALGCLVKDYFPEPVTVSWNSGALTSGVHTFPAVLQSSGLYSLSSVVTVPSSSLGTQTYICNVNHKPSNTKVDKKVEPKSCDKTHTCPPCPAPEAAGGPSVFLFPPKPKDTLMISRTPEVTCVVVDVSHEDPEVKFNWYVDGVEVHNAKTKPREEQYNSTYRVVSVLTVLHQDWLNGKEYKCKVSNKALPAPIEKTISKAKGQPREPQVYTLPPSREEMTKNQVSLTCLVKGFYPSDIAVEWESNGQPENNYKTTPPVLDSDGSFFLYSKLTVDKSRWQQGNVFSCSVMHEALHNHYTQKSLSLSPGQGQDRHMIRMRQLIDIVDQLKNYVNDLVPEFLPAPENVTTNCEWSAFSCFQKAQLKSANTGNNERIINVSIKKLKRKPPSTNAGRRQKHRLTCPSCDSYEKKPPKEFLERFKSLLQKMIHQHLSSRTHGSEDS

SEQ ID NO: 49 - protein, 579 aa, Artificial
  Synthetic sequence
QVQLVQSGAEVKKPGSSVKVSCKASGGTFSSYAISWVRQAPGQGLEWMGLIIPMFDTAGYAQKFQGRVAITVDESTSTAYMELSSLRSEDTAVYYCARAEHSSTGTFDYWGQGTLVTVSSASTKGPSVFPLAPSSKSTSGGTAALGCLVKDYFPEPVTVSWNSGALTSGVHTFPAVLQSSGLYSLSSVVTVPSSSLGTQTYICNVNHKPSNTKVDKKVEPKSCDKTHTCPPCPAPEAAGGPSVFLFPPKPKDTLMISRTPEVTCVVVDVSHEDPEVKFNWYVDGVEVHNAKTKPREEQYNSTYRVVSVLTVLHQDWLNGKEYKCKVSNKALPAPIEKTISKAKGQPREPQVYTLPPSREEMTKNQVSLTCLVKGFYPSDIAVEWESNGQPENNYKTTPPVLDSDGSFFLYSKLTVDKSRWQQGNVFSCSVMHEALHNHYTQKSLSLSPGQGQDRHMIRMRQLIDIVDQLKNYVNDLVPEFLPAPEDVETNCEWSAFSCFQKAQLKSANTGNNERIINVSIKKLKRKPPSTNAGKHRLTCPSCDSYEKKPPKEFLERFKSLLQKMIHQHLSSRTHGSEDS

SEQ ID NO: 50 - protein, 580 aa, Artificial
  Synthetic sequence
QVQLVQSGAEVKKPGSSVKVSCKASGGTFSSYAISWVRQAPGQGLEWMGLIIPMFDTAGYAQKFQGRVAITVDESTSTAYMELSSLRSEDTAVYYCARAEHSSTGTFDYWGQGTLVTVSSASTKGPSVFPLAPSSKSTSGGTAALGCLVKDYFPEPVTVSWNSGALTSGVHTFPAVLQSSGLYSLSSVVTVPSSSLGTQTYICNVNHKPSNTKVDKKVEPKSCDKTHTCPPCPAPEAAGGPSVFLFPPKPKDTLMISRTPEVTCVVVDVSHEDPEVKFNWYVDGVEVHNAKTKPREEQYNSTYRVVSVLTVLHQDWLNGKEYKCKVSNKALPAPIEKTISKAKGQPREPQVYTLPPSREEMTKNQVSLTCLVKGFYPSDIAVEWESNGQPENNYKTTPPVLDSDGSFFLYSKLTVDKSRWQQGNVFSCSVMHEALHNHYTQKSLSLSPGQGQDRHMIRMRQLIDIVDQLKNYVNDLVPEFLPAPEDVETNCEWSAFSCFQKAQLKSANTGNNERIINVSIKKLKRKSTNAGRRQKHRLTCPSCDSYEKKPPKEFLERFKSLLQKMIHQHLSSRTHGSEDS

SEQ ID NO: 51 - protein, 582 aa, Artificial
  Synthetic sequence
QVQLVQSGAEVKKPGSSVKVSCKASGGTFSSYAISWVRQAPGQGLEWMGLIIPMFDTAGYAQKFQGRVAITVDESTSTAYMELSSLRSEDTAVYYCARAEHSSTGTFDYWGQGTLVTVSSASTKGPSVFPLAPSSKSTSGGTAALGCLVKDYFPEPVTVSWNSGALTSGVHTFPAVLQSSGLYSLSSVVTVPSSSLGTQTYICNVNHKPSNTKVDKKVEPKSCDKTHTCPPCPAPEAAGGPSVFLFPPKPKDTLMISRTPEVTCVVVDVSHEDPEVKFNWYVDGVEVHNAKTKPREEQYNSTYRVVSVLTVLHQDWLNGKEYKCKVSNKALPAPIEKTISKAKGQPREPQVYTLPPSREEMTKNQVSLTCLVKGFYPSDIAVEWESNGQPENNYKTTPPVLDSDGSFFLYSKLTVDKSRWQQGNVFSCSVMHEALHNHYTQKSLSLSPGHKSDITLQEMRQLIDIVDQLKNYVNDLVPEFLPAPEDVETNCEWSAFSCFQKAQLKSANTGNNERIINVSIKKLKRKPPSTNAGRRQKHRLTCPSCDSYEKKPPKEFLERFKSLLQKMIHQHLSSRTHGSEDS

SEQ ID NO: 52 - protein, 582 aa, Artificial
  Synthetic sequence
QVQLVQSGAEVKKPGSSVKVSCKASGGTFSSYAISWVRQAPGQGLEWMGLIIPMFDTAGYAQKFQGRVAITVDESTSTAYMELSSLRSEDTAVYYCARAEHSSTGTFDYWGQGTLVTVSSASTKGPSVFPLAPSSKSTSGGTAALGCLVKDYFPEPVTVSWNSGALTSGVHTFPAVLQSSGLYSLSSVVTVPSSSLGTQTYICNVNHKPSNTKVDKKVEPKSCDKTHTCPPCPAPEAAGGPSVFLFPPKPKDTLMISRTPEVTCVVVDVSHEDPEVKFNWYVDGVEVHNAKTKPREEQYNSTYRVVSVLTVLHQDWLNGKEYKCKVSNKALPAPIEKTISKAKGQPREPQVYTLPPSREEMTKNQVSLTCLVKGFYPSDIAVEWESNGQPENNYKTTPPVLDSDGSFFLYSKLTVDKSRWQQGNVFSCSVMHEALHNHYTQKSLSLSPGQGQDRHMIRMRQLIDIVDQLKNYVNDLVPEFLPAPEDVETNCEWSAFSCFQKAQLKSANTGNNERIINVSIEKLKRKPPSTNAGRRQKHRLTCPSCDSYEKKPPKEFLERFKSLLQKMIHQHLSSRTHGSEDS

SEQ ID NO: 53 - protein, 582 aa, Artificial
  Synthetic sequence
QVQLVQSGAEVKKPGSSVKVSCKASGGTFSSYAISWVRQAPGQGLEWMGLIIPMFDTAGYAQKFQGRVAITVDESTSTAYMELSSLRSEDTAVYYCARAEHSSTGTFDYWGQGTLVTVSSASTKGPSVFPLAPSSKSTSGGTAALGCLVKDYFPEPVTVSWNSGALTSGVHTFPAVLQSSGLYSLSSVVTVPSSSLGTQTYICNVNHKPSNTKVDKKVEPKSCDKTHTCPPCPAPEAAGGPSVFLFPPKPKDTLMISRTPEVTCVVVDVSHEDPEVKFNWYVDGVEVHNAKTKPREEQYNSTYRVVSVLTVLHQDWLNGKEYKCKVSNKALPAPIEKTISKAKGQPREPQVYTLPPSREEMTKNQVSLTCLVKGFYPSDIAVEWESNGQPENNYKTTPPVLDSDGSFFLYSKLTVDKSRWQQGNVFSCSVMHEALHNHYTQKSLSLSPGQGQDRHMQRMRQLIDIVDQLKNYVNDLVPEFLPAPEDVETNCEWSAFSCFQKAQLKSANTGNNERIINVSIKKLKRKPESTNAGRRQKHRLTCPSCDSYEKKPPKEFLERFKSLLQKMIHQHLSSRTHGSEDS

SEQ ID NO: 54 - protein, 582 aa, Artificial
  Synthetic sequence
QVQLVQSGAEVKKPGSSVKVSCKASGGTFSSYAISWVRQAPGQGLEWMGLIIPMFDTAGYAQKFQGRVAITVDESTSTAYMELSSLRSEDTAVYYCARAEHSSTGTFDYWGQGTLVTVSSASTKGPSVFPLAPSSKSTSGGTAALGCLVKDYFPEPVTVSWNSGALTSGVHTFPAVLQSSGLYSLSSVVTVPSSSLGTQTYICNVNHKPSNTKVDKKVEPKSCDKTHTCPPCPAPEAAGGPSVFLFPPKPKDTLMISRTPEVTCVVVDVSHEDPEVKFNWYVDGVEVHNAKTKPREEQYNSTYRVVSVLTVLHQDWLNGKEYKCKVSNKALPAPIEKTISKAKGQPREPQVYTLPPSREEMTKNQVSLTCLVKGFYPSDIAVEWESNGQPENNYKTTPPVLDSDGSFFLYSKLTVDKSRWQQGNVFSCSVMHEALHNHYTQKSLSLSPGQGQDRHMIRMRQLIDIVDQLKNYVNDLVPEFLPAPEDVETNCEWSAFSCFQKAQLKSANTGNNERIINVSIKKLKRDAPSTNAGRRQKHRLTCPSCDSYEKKPPKEFLERFKSLLQKMIHQHLSSRTHGSEDS

SEQ ID NO: 55 - protein, 597 aa, Artificial
  Synthetic sequence
QVQLVQSGAEVKKPGSSVKVSCKASGGTFSSYAISWVRQAPGQGLEWMGLIIPMFDTAGYAQKFQGRVAITVDESTSTAYMELSSLRSEDTAVYYCARAEHSSTGTFDYWGQGTLVTVSSASTKGPSVFPLAPSSKSTSGGTAALGCLVKDYFPEPVTVSWNSGALTSGVHTFPAVLQSSGLYSLSSVVTVPSSSLGTQTYICNVNHKPSNTKVDKKVEPKSCDKTHTCPPCPAPEAAGGPSVFLFPPKPKDTLMISRTPEVTCVVVDVSHEDPEVKFNWYVDGVEVHNAKTKPREEQYNSTYRVVSVLTVLHQDWLNGKEYKCKVSNKALPAPIEKTISKAKGQPREPQVYTLPPCRDELTKNQVSLWCLVKGFYPSDIAVEWESNGQPENNYKTTPPVLDSDGSFFLYSKLTVDKSRWQQGNVFSCSVMHEALHNHYTQKSLSLSPGGGGGSGGGGSGGGGSHKSDITLQEMRQLIDIVDQLKNYVNDLVPEFLPAPEDVETNCEWSAFSCFQKAQLKSANTGNNERIINVSIKKLKRKPPSTNAGRRQKHRLTCPSCDSYEKKPPKEFLERFKSLLQKMIHQHLSSRTHGSEDS

SEQ ID NO: 56 - protein, 597 aa, Artificial
  Synthetic sequence
QVQLVQSGAEVKKPGSSVKVSCKASGGTFSSYAISWVRQAPGQGLEWMGLIIPMFDTAGYAQKFQGRVAITVDESTSTAYMELSSLRSEDTAVYYCARAEHSSTGTFDYWGQGTLVTVSSASTKGPSVFPLAPSSKSTSGGTAALGCLVKDYFPEPVTVSWNSGALTSGVHTFPAVLQSSGLYSLSSVVTVPSSSLGTQTYICNVNHKPSNTKVDKKVEPKSCDKTHTCPPCPAPEAAGGPSVFLFPPKPKDTLMISRTPEVTCVVVDVSHEDPEVKFNWYVDGVEVHNAKTKPREEQYNSTYRVVSVLTVLHQDWLNGKEYKCKVSNKALPAPIEKTISKAKGQPREPQVYTLPPCRDELTKNQVSLWCLVKGFYPSDIAVEWESNGQPENNYKTTPPVLDSDGSFFLYSKLTVDKSRWQQGNVFSCSVMHEALHNHYTQKSLSLSPGGGGGSGGGGSGGGGSHKSDITLQEIIKTLNIVDQLKNYVNDLVPEFLPAPEDVETNCEWSAFSCFQKAQLKSANTGNNERIINVSIKKLKRKPPSTNAGRRQKHRLTCPSCDSYEKKPPKEFLERFKSLLQKMIHQHLSSRTHGSEDS

SEQ ID NO: 57 - protein, 597 aa, Artificial
  Synthetic sequence
QVQLVQSGAEVKKPGSSVKVSCKASGGTFSSYAISWVRQAPGQGLEWMGLIIPMFDTAGYAQKFQGRVAITVDESTSTAYMELSSLRSEDTAVYYCARAEHSSTGTFDYWGQGTLVTVSSASTKGPSVFPLAPSSKSTSGGTAALGCLVKDYFPEPVTVSWNSGALTSGVHTFPAVLQSSGLYSLSSVVTVPSSSLGTQTYICNVNHKPSNTKVDKKVEPKSCDKTHTCPPCPAPEAAGGPSVFLFPPKPKDTLMISRTPEVTCVVVDVSHEDPEVKFNWYVDGVEVHNAKTKPREEQYNSTYRVVSVLTVLHQDWLNGKEYKCKVSNKALPAPIEKTISKAKGQPREPQVYTLPPCRDELTKNQVSLWCLVKGFYPSDIAVEWESNGQPENNYKTTPPVLDSDGSFFLYSKLTVDKSRWQQGNVFSCSVMHEALHNHYTQKSLSLSPGGGGGSGGGGSGGGGSHKSDITLQEIIKLIDIVDQLKNYVNDLVPEFLPAPEDVETNCEWSAFSCFQKAQLKSANTGNNERIINVSIKKLKRKPPSTNAGRRQKHRLTCPSCDSYEKKPPKEFLERFKSLLQKMIHQHLSSRTHGSEDS

SEQ ID NO: 58 - protein, 597 aa, Artificial
  Synthetic sequence
QVQLVQSGAEVKKPGSSVKVSCKASGGTFSSYAISWVRQAPGQGLEWMGLIIPMFDTAGYAQKFQGRVAITVDESTSTAYMELSSLRSEDTAVYYCARAEHSSTGTFDYWGQGTLVTVSSASTKGPSVFPLAPSSKSTSGGTAALGCLVKDYFPEPVTVSWNSGALTSGVHTFPAVLQSSGLYSLSSVVTVPSSSLGTQTYICNVNHKPSNTKVDKKVEPKSCDKTHTCPPCPAPEAAGGPSVFLFPPKPKDTLMISRTPEVTCVVVDVSHEDPEVKFNWYVDGVEVHNAKTKPREEQYNSTYRVVSVLTVLHQDWLNGKEYKCKVSNKALPAPIEKTISKAKGQPREPQVYTLPPCRDELTKNQVSLWCLVKGFYPSDIAVEWESNGQPENNYKTTPPVLDSDGSFFLYSKLTVDKSRWQQGNVFSCSVMHEALHNHYTQKSLSLSPGGGGGSGGGGSGGGGSHKSDITLQEIIQLIDIVDQLKNYVNDLVPEFLPAPEDVETNCEWSAFSCFQKAQLKSANTGNNERIINVSIKKLKRKPPSTNAGRRQKHRLTCPSCDSYEKKPPKEFLERFKSLLQKMIHQHLSSRTHGSEDS

SEQ ID NO: 59 - protein, 595 aa, Artificial
  Synthetic sequence
QVQLVQSGAEVKKPGSSVKVSCKASGGTFSSYAISWVRQAPGQGLEWMGLIIPMFDTAGYAQKFQGRVAITVDESTSTAYMELSSLRSEDTAVYYCARAEHSSTGTFDYWGQGTLVTVSSASTKGPSVFPLAPSSKSTSGGTAALGCLVKDYFPEPVTVSWNSGALTSGVHTFPAVLQSSGLYSLSSVVTVPSSSLGTQTYICNVNHKPSNTKVDKKVEPKSCDKTHTCPPCPAPEAAGGPSVFLFPPKPKDTLMISRTPEVTCVVVDVSHEDPEVKFNWYVDGVEVHNAKTKPREEQYNSTYRVVSVLTVLHQDWLNGKEYKCKVSNKALPAPIEKTISKAKGQPREPQVYTLPPCRDELTKNQVSLWCLVKGFYPSDIAVEWESNGQPENNYKTTPPVLDSDGSFFLYSKLTVDKSRWQQGNVFSCSVMHEALHNHYTQKSLSLSPGGGGGSGGGGSGGGGSHKSDITLQEMRQLIDIVDQLKNYVNDLVPEFLPAPEDVETNCEWSAFSCFQKAQLKSANTGNNERIINVSIKKLKRKSTNAGRRQKHRLTCPSCDSYEKKPPKEFLERFKSLLQKMIHQHLSSRTHGSEDS

SEQ ID NO: 60 - protein, 588 aa, Artificial
  Synthetic sequence
QVQLVQSGAEVKKPGSSVKVSCKASGGTFSSYAISWVRQAPGQGLEWMGLIIPMFDTAGYAQKFQGRVAITVDESTSTAYMELSSLRSEDTAVYYCARAEHSSTGTFDYWGQGTLVTVSSASTKGPSVFPLAPSSKSTSGGTAALGCLVKDYFPEPVTVSWNSGALTSGVHTFPAVLQSSGLYSLSSVVTVPSSSLGTQTYICNVNHKPSNTKVDKKVEPKSCDKTHTCPPCPAPEAAGGPSVFLFPPKPKDTLMISRTPEVTCVVVDVSHEDPEVKFNWYVDGVEVHNAKTKPREEQYNSTYRVVSVLTVLHQDWLNGKEYKCKVSNKALPAPIEKTISKAKGQPREPQVYTLPPCRDELTKNQVSLWCLVKGFYPSDIAVEWESNGQPENNYKTTPPVLDSDGSFFLYSKLTVDKSRWQQGNVFSCSVMHEALHNHYTQKSLSLSPGGGGGSGGGGSGGGGSMRQLIDIVDQLKNYVNDLVPEFLPAPEDVETNCEWSAFSCFQKAQLKSANTGNNERIINVSIKKLKRKPPSTNAGRRQKHRLTCPSCDSYEKKPPKEFLERFKSLLQKMIHQHLSSRTHGSEDS

SEQ ID NO: 61 - protein, 588 aa, Artificial
  Synthetic sequence
QVQLVQSGAEVKKPGSSVKVSCKASGGTFSSYAISWVRQAPGQGLEWMGLIIPMFDTAGYAQKFQGRVAITVDESTSTAYMELSSLRSEDTAVYYCARAEHSSTGTFDYWGQGTLVTVSSASTKGPSVFPLAPSSKSTSGGTAALGCLVKDYFPEPVTVSWNSGALTSGVHTFPAVLQSSGLYSLSSVVTVPSSSLGTQTYICNVNHKPSNTKVDKKVEPKSCDKTHTCPPCPAPEAAGGPSVFLFPPKPKDTLMISRTPEVTCVVVDVSHEDPEVKFNWYVDGVEVHNAKTKPREEQYNSTYRVVSVLTVLHQDWLNGKEYKCKVSNKALPAPIEKTISKAKGQPREPQVYTLPPCRDELTKNQVSLWCLVKGFYPSDIAVEWESNGQPENNYKTTPPVLDSDGSFFLYSKLTVDKSRWQQGNVFSCSVMHEALHNHYTQKSLSLSPGGGGGSGGGGSGGGGSMRQLIDIVDNLTNYVNDLVPEFLPAPEDVETNCEWSAFSCFQKAQLKSANTGNNERIINVSIKKLKRKPPSTNAGRRQKHRLTCPSCDSYEKKPPKEFLERFKSLLQKMIHQHLSSRTHGSEDS

SEQ ID NO: 62 - protein, 586 aa, Artificial
  Synthetic sequence
QVQLVQSGAEVKKPGSSVKVSCKASGGTFSSYAISWVRQAPGQGLEWMGLIIPMFDTAGYAQKFQGRVAITVDESTSTAYMELSSLRSEDTAVYYCARAEHSSTGTFDYWGQGTLVTVSSASTKGPSVFPLAPSSKSTSGGTAALGCLVKDYFPEPVTVSWNSGALTSGVHTFPAVLQSSGLYSLSSVVTVPSSSLGTQTYICNVNHKPSNTKVDKKVEPKSCDKTHTCPPCPAPEAAGGPSVFLFPPKPKDTLMISRTPEVTCVVVDVSHEDPEVKFNWYVDGVEVHNAKTKPREEQYNSTYRVVSVLTVLHQDWLNGKEYKCKVSNKALPAPIEKTISKAKGQPREPQVYTLPPCRDELTKNQVSLWCLVKGFYPSDIAVEWESNGQPENNYKTTPPVLDSDGSFFLYSKLTVDKSRWQQGNVFSCSVMHEALHNHYTQKSLSLSPGGGGGSGGGGSGGGGSMRQLIDIVDQLKNYVNDLVPEFLPAPEDVETNCEWSAFSCFQKAQLKSANTGNNERIINVSIKKLKRKSTNAGRRQKHRLTCPSCDSYEKKPPKEFLERFKSLLQKMIHQHLSSRTHGSEDS

SEQ ID NO: 63 - protein, 589 aa, Artificial
  Synthetic sequence
QVQLVQSGAEVKKPGSSVKVSCKASGGTFSSYAISWVRQAPGQGLEWMGLIIPMFDTAGYAQKFQGRVAITVDESTSTAYMELSSLRSEDTAVYYCARAEHSSTGTFDYWGQGTLVTVSSASTKGPSVFPLAPSSKSTSGGTAALGCLVKDYFPEPVTVSWNSGALTSGVHTFPAVLQSSGLYSLSSVVTVPSSSLGTQTYICNVNHKPSNTKVDKKVEPKSCDKTHTCPPCPAPEAAGGPSVFLFPPKPKDTLMISRTPEVTCVVVDVSHEDPEVKFNWYVDGVEVHNAKTKPREEQYNSTYRVVSVLTVLHQDWLNGKEYKCKVSNKALPAPIEKTISKAKGQPREPQVYTLPPCRDELTKNQVSLWCLVKGFYPSDIAVEWESNGQPENNYKTTPPVLDSDGSFFLYSKLTVDKSRWQQGNVFSCSVMHEALHNHYTQKSLSLSPGGGGGSGGGGSGGGGSQGQDRHMIRMRQLIDIVDNLTNYVNDLVPEFLPAPEDVETNAEWSAFSCFQKAQLKSANTGNNERIINVSIKKLKRKPPSTNATTPSCDSYEKKPPKEFLERFKSLLQKMIHQHLSSRTHGSEDS

SEQ ID NO: 64 - protein, 599 aa, Artificial
  Synthetic sequence
QVQLVQSGAEVKKPGSSVKVSCKASGGTFSSYAISWVRQAPGQGLEWMGLIIPMFDTAGYAQKFQGRVAITVDESTSTAYMELSSLRSEDTAVYYCARAEHSSTGTFDYWGQGTLVTVSSASTKGPSVFPLAPSSKSTSGGTAALGCLVKDYFPEPVTVSWNSGALTSGVHTFPAVLQSSGLYSLSSVVTVPSSSLGTQTYICNVNHKPSNTKVDKKVEPKSCDKTHTCPPCPAPEAAGGPSVFLFPPKPKDTLMISRTPEVTCVVVDVSHEDPEVKFNWYVDGVEVHNAKTKPREEQYNSTYRVVSVLTVLHQDWLNGKEYKCKVSNKALPAPIEKTISKAKGQPREPQVYTLPPCRDELTKNQVSLWCLVKGFYPSDIAVEWESNGQPENNYKTTPPVLDSDGSFFLYSKLTVDKSRWQQGNVFSCSVMHEALHNHYTQKSLSLSPGGGGGSGGGGSGGGGSHKSDITLQEIIMRQLIDIVDQLKNYVNDLVPEFLPAPEDVETNCEWSAFSCFQKAQLKSANTGNNERIINVSIKKLKRKPPSTNAGRRQKHRLTCPSCDSYEKKPPKEFLERFKSLLQKMIHQHLSSRTHGSEDS

SEQ ID NO: 65 - protein, 597 aa, Artificial
  Synthetic sequence
QVQLVQSGAEVKKPGSSVKVSCKASGGTFSSYAISWVRQAPGQGLEWMGLIIPMFDTAGYAQKFQGRVAITVDESTSTAYMELSSLRSEDTAVYYCARAEHSSTGTFDYWGQGTLVTVSSASTKGPSVFPLAPSSKSTSGGTAALGCLVKDYFPEPVTVSWNSGALTSGVHTFPAVLQSSGLYSLSSVVTVPSSSLGTQTYICNVNHKPSNTKVDKKVEPKSCDKTHTCPPCPAPEAAGGPSVFLFPPKPKDTLMISRTPEVTCVVVDVSHEDPEVKFNWYVDGVEVHNAKTKPREEQYNSTYRVVSVLTVLHQDWLNGKEYKCKVSNKALPAPIEKTISKAKGQPREPQVYTLPPCRDELTKNQVSLWCLVKGFYPSDIAVEWESNGQPENNYKTTPPVLDSDGSFFLYSKLTVDKSRWQQGNVFSCSVMHEALHNHYTQKSLSLSPGGGGGSGGGGSGGGGSHKSDITLQEMRQLIDIVDQLKNYVNDLVPEFLPAPEDVETNCEWSAFSCFQKAQLKSANTGNNERIINVSIKKLKRKPPSTNAGRRQKHRLTCPSCDSYEKKPPKEFLERFKSLLQNMTHQHLSSRTHGSEDS

SEQ ID NO: 66 - protein, 597 aa, Artificial
  Synthetic sequence
QVQLVQSGAEVKKPGSSVKVSCKASGGTFSSYAISWVRQAPGQGLEWMGLIIPMFDTAGYAQKFQGRVAITVDESTSTAYMELSSLRSEDTAVYYCARAEHSSTGTFDYWGQGTLVTVSSASTKGPSVFPLAPSSKSTSGGTAALGCLVKDYFPEPVTVSWNSGALTSGVHTFPAVLQSSGLYSLSSVVTVPSSSLGTQTYICNVNHKPSNTKVDKKVEPKSCDKTHTCPPCPAPEAAGGPSVFLFPPKPKDTLMISRTPEVTCVVVDVSHEDPEVKFNWYVDGVEVHNAKTKPREEQYNSTYRVVSVLTVLHQDWLNGKEYKCKVSNKALPAPIEKTISKAKGQPREPQVYTLPPCRDELTKNQVSLWCLVKGFYPSDIAVEWESNGQPENNYKTTPPVLDSDGSFFLYSKLTVDKSRWQQGNVFSCSVMHEALHNHYTQKSLSLSPGGGGGSGGGGSGGGGSHKSDITLQEMRQLIDIVDQLKNYVNDLVPEFLPAPENVTTNCEWSAFSCFQKAQLKSANTGNNERIINVSIKKLKRKPPSTNAGRRQKHRLTCPSCDSYEKKPPKEFLERFKSLLQKMIHQHLSSRTHGSEDS

SEQ ID NO: 67 - protein, 597 aa, Artificial
  Synthetic sequence
QVQLVQSGAEVKKPGSSVKVSCKASGGTFSSYAISWVRQAPGQGLEWMGLIIPMFDTAGYAQKFQGRVAITVDESTSTAYMELSSLRSEDTAVYYCARAEHSSTGTFDYWGQGTLVTVSSASTKGPSVFPLAPSSKSTSGGTAALGCLVKDYFPEPVTVSWNSGALTSGVHTFPAVLQSSGLYSLSSVVTVPSSSLGTQTYICNVNHKPSNTKVDKKVEPKSCDKTHTCPPCPAPEAAGGPSVFLFPPKPKDTLMISRTPEVTCVVVDVSHEDPEVKFNWYVDGVEVHNAKTKPREEQYNSTYRVVSVLTVLHQDWLNGKEYKCKVSNKALPAPIEKTISKAKGQPREPQVYTLPPCRDELTKNQVSLWCLVKGFYPSDIAVEWESNGQPENNYKTTPPVLDSDGSFFLYSKLTVDKSRWQQGNVFSCSVMHEALHNHYTQKSLSLSPGGGGGSGGGGSGGGGSHKSDITLQEMRQLINITDQLKNYVNDLVPEFLPAPEDVETNCEWSAFSCFQKAQLKSANTGNNERIINVSIKKLKRKPPSTNAGRRQKHRLTCPSCDSYEKKPPKEFLERFKSLLQKMIHQHLSSRTHGSEDS

SEQ ID NO: 68 - protein, 582 aa, Artificial
  Synthetic sequence
QVQLVQSGAEVKKPGSSVKVSCKASGGTFSSYAISWVRQAPGQGLEWMGLIIPMFDTAGYAQKFQGRVAITVDESTSTAYMELSSLRSEDTAVYYCARAEHSSTGTFDYWGQGTLVTVSSASTKGPSVFPLAPSSKSTSGGTAALGCLVKDYFPEPVTVSWNSGALTSGVHTFPAVLQSSGLYSLSSVVTVPSSSLGTQTYICNVNHKPSNTKVDKKVEPKSCDKTHTCPPCPAPEAAGGPSVFLFPPKPKDTLMISRTPEVTCVVVDVSHEDPEVKFNWYVDGVEVHNAKTKPREEQYNSTYRVVSVLTVLHQDWLNGKEYKCKVSNKALPAPIEKTISKAKGQPREPQVYTLPPCRDELTKNQVSLWCLVKGFYPSDIAVEWESNGQPENNYKTTPPVLDSDGSFFLYSKLTVDKSRWQQGNVFSCSVMHEALHNHYTQKSLSLSPGQGQDQHMIRMRQLIDIVDQLKNYVNDLVPEFLPAPEDVETNCEWSAFSCFQKAQLKSANTGNNERIINVSIKKLKEKPPSTNAGRRQKHRLTCPSCDSYEKKPPKEFLERFKSLLQKMIHQHLSSRTHGSEDS

SEQ ID NO: 69 - protein, 10 aa, Artificial
  Synthetic sequence
GGGGSGGGGS

SEQ ID NO: 70 - protein, 227 aa, Artificial
  Synthetic sequence
DKTHTCPPCPAPEAAGGPSVFLFPPKPKDTLMISRTPEVTCVVVDVSHEDPEVKFNWYVDGVEVHNAKTKPREEQYNSTYRVVSVLTVLHQDWLNGKEYKCKVSNKALPAPIEKTISKAKGQPREPQVYTLPPSREEMTKNQVSLTCLVKGFYPSDIAVEWESNGQPENNYKTTPPVLDSDGSFFLYSKLTVDKSRWQQGNVFSCSVMHEALHNHYTQKSLSLSPGK

SEQ ID NO: 71 - protein, 449 aa, Artificial
  Synthetic sequence
QVQLVQSGAEVKKPGSSVKVSCKASGGTFSSYAISWVRQAPGQGLEWMGLIIPMFDTAGYAQKFQGRVAITVDESTSTAYMELSSLRSEDTAVYYCARAEHSSTGTFDYWGQGTLVTVSSASTKGPSVFPLAPSSKSTSGGTAALGCLVKDYFPEPVTVSWNSGALTSGVHTFPAVLQSSGLYSLSSVVTVPSSSLGTQTYICNVNHKPSNTKVDKKVEPKSCDKTHTCPPCPAPEAAGGPSVFLFPPKPKDTLMISRTPEVTCVVVDVSHEDPEVKFNWYVDGVEVHNAKTKPREEQYNSTYRVVSVLTVLHQDWLNGKEYKCKVSNKALPAPIEKTISKAKGQPREPQVYTLPPSREEMTKNQVSLTCLVKGFYPSDIAVEWESNGQPENNYKTTPPVLDSDGSFFLYSKLTVDKSRWQQGNVFSCSVMHEALHNHYTQKSLSLSPG

SEQ ID NO: 72 - protein, 15 aa, Artificial
  Synthetic sequence
GGGGSGGGGSGGGGS

SEQ ID NO: 73 - protein, 449 aa, Artificial
  Synthetic sequence
QVQLVQSGAEVKKPGSSVKVSCKASGGTFSSYAISWVRQAPGQGLEWMGLIIPMFDTAGYAQKFQGRVAITVDESTSTAYMELSSLRSEDTAVYYCARAEHSSTGTFDYWGQGTLVTVSSASTKGPSVFPLAPSSKSTSGGTAALGCLVKDYFPEPVTVSWNSGALTSGVHTFPAVLQSSGLYSLSSVVTVPSSSLGTQTYICNVNHKPSNTKVDKKVEPKSCDKTHTCPPCPAPEAAGGPSVFLFPPKPKDTLMISRTPEVTCVVVDVSHEDPEVKFNWYVDGVEVHNAKTKPREEQYNSTYRVVSVLTVLHQDWLNGKEYKCKVSNKALPAPIEKTISKAKGQPREPQVYTLPPCRDELTKNQVSLWCLVKGFYPSDIAVEWESNGQPENNYKTTPPVLDSDGSFFLYSKLTVDKSRWQQGNVFSCSVMHEALHNHYTQKSLSLSPG

SEQ ID NO: 74 - protein, 133 aa, Artificial [sequence omitted]

SEQ ID NO: 75 - protein, 133 aa, Artificial
  Synthetic sequence
HKSDIHMIRMRQLIDIVDQLKNYVNDLVPEFLPAPEDVETNCEWSAFSCFQKAQLKSANTGNNERIINVSIKKLKRKPPSTNAGRRQKHRLTCPSCDSYEKKPPKEFLERFKSLLQKMIHQHLSSRTHGSEDS

SEQ ID NO: 76 - protein, 133 aa, Artificial
  Synthetic sequence
HKCDIHMIRMRQLIDIVDQLKNYVNDLVPEFLPAPEDVETNCEWSAFSCFQKAQLKSANTGNNERIINVSIKKLKRKPPSTNAGRRQKHRLTCPSCDSYEKKPPKEFLERFKSLLQKMIHQHCSSRTHGSEDS

SEQ ID NO: 77 - protein, 133 aa, Artificial
  Synthetic sequence
HKSDITLQEMRQLIDIVDQLKNYVNDLVPEFLPAPEDVETNCEWSAFSCFQKAQLKSANTGNNERIINVSIKKLKRKPPSTNAGRRQKHRLTCPSCDSYEKKPPKEFLERFKSLLQKMIHQHLSSRTHGSEDS

SEQ ID NO: 78 - protein, 133 aa, Artificial
  Synthetic sequence
HKSDITLQEIIKTLNIVDQLKNYVNDLVPEFLPAPEDVETNCEWSAFSCFQKAQLKSANTGNNERIINVSIKKLKRKPPSTNAGRRQKHRLTCPSCDSYEKKPPKEFLERFKSLLQKMIHQHLSSRTHGSEDS

SEQ ID NO: 79 - protein, 133 aa, Artificial
  Synthetic sequence
HKSDITLQEIIKLIDIVDQLKNYVNDLVPEFLPAPEDVETNCEWSAFSCFQKAQLKSANTGNNERIINVSIKKLKRKPPSTNAGRRQKHRLTCPSCDSYEKKPPKEFLERFKSLLQKMIHQHLSSRTHGSEDS

SEQ ID NO: 80 - protein, 133 aa, Artificial
  Synthetic sequence
HKSDITLQEIIQLIDIVDQLKNYVNDLVPEFLPAPEDVETNCEWSAFSCFQKAQLKSANTGNNERIINVSIKKLKRKPPSTNAGRRQKHRLTCPSCDSYEKKPPKEFLERFKSLLQKMIHQHLSSRTHGSEDS

SEQ ID NO: 81 - protein, 135 aa, Artificial
  Synthetic sequence
HKSDITLQEIIMRQLIDIVDQLKNYVNDLVPEFLPAPEDVETNCEWSAFSCFQKAQLKSANTGNNERIINVSIKKLKRKPPSTNAGRRQKHRLTCPSCDSYEKKPPKEFLERFKSLLQKMIHQHLSSRTHGSEDS

SEQ ID NO: 82 - protein, 133 aa, Artificial
  Synthetic sequence
QGQNRTMIRMRQLIDIVDQLKNYVNDLVPEFLPAPEDVETNCEWSAFSCFQKAQLKSANTGNNERIINVSIKKLKRKPPSTNAGRRQKHRLTCPSCDSYEKKPPKEFLERFKSLLQKMIHQHLSSRTHGSEDS

SEQ ID NO: 83 - protein, 133 aa, Artificial
  Synthetic sequence
QGQDNHTIRMRQLIDIVDQLKNYVNDLVPEFLPAPEDVETNCEWSAFSCFQKAQLKSANTGNNERIINVSIKKLKRKPPSTNAGRRQKHRLTCPSCDSYEKKPPKEFLERFKSLLQKMIHQHLSSRTHGSEDS

SEQ ID NO: 84 - protein, 133 aa, Artificial
  Synthetic sequence
QGQDRHMIRMRQLINITDQLKNYVNDLVPEFLPAPEDVETNCEWSAFSCFQKAQLKSANTGNNERIINVSIKKLKRKPPSTNAGRRQKHRLTCPSCDSYEKKPPKEFLERFKSLLQKMIHQHLSSRTHGSEDS

SEQ ID NO: 85 - protein, 133 aa, Artificial
  Synthetic sequence
QGQDRHMIRMRQLIDIVDNLTNYVNDLVPEFLPAPEDVETNCEWSAFSCFQKAQLKSANTGNNERIINVSIKKLKRKPPSTNAGRRQKHRLTCPSCDSYEKKPPKEFLERFKSLLQKMIHQHLSSRTHGSEDS

SEQ ID NO: 86 - protein, 133 aa, Artificial
  Synthetic sequence
QGQDRHMIRMRQLIDIVDQLKNYVNDLVPEFLPAPEDVETNCEWSAFSCFQKAQLKSANTGNNERIINVSIKKLKNKTPSTNAGRRQKHRLTCPSCDSYEKKPPKEFLERFKSLLQKMIHQHLSSRTHGSEDS

SEQ ID NO: 87 - protein, 133 aa, Artificial
  Synthetic sequence
QGQDRHMIRMRQLIDIVDQLKNYVNDLVPEFLPAPEDVETNCEWSAFSCFQKAQLKSANTGNNERIINVSIKKLKRNSTSTNAGRRQKHRLTCPSCDSYEKKPPKEFLERFKSLLQKMIHQHLSSRTHGSEDS

SEQ ID NO: 88 - protein, 133 aa, Artificial
  Synthetic sequence
QGQDRHMIRMRQLIDIVDQLKNYVNDLVPEFLPAPEDVETNCEWSAFSCFQKAQLKSANTGNNERIINVSIKKLKRKPNSTNAGRRQKHRLTCPSCDSYEKKPPKEFLERFKSLLQKMIHQHLSSRTHGSEDS

SEQ ID NO: 89 - protein, 133 aa, Artificial
  Synthetic sequence
QGQDRHMIRMRQLIDIVDQLKNYVNDLVPEFLPAPEDVETNCEWSAFSCFQKAQLKSANTGNNERIINVSIKKLKRKPPNTTAGRRQKHRLTCPSCDSYEKKPPKEFLERFKSLLQKMIHQHLSSRTHGSEDS

SEQ ID NO: 90 - protein, 133 aa, Artificial
  Synthetic sequence
QGQDRHMIRMRQLIDIVDQLKNYVNDLVPEFLPAPEDVETNCEWSAFSCFQKAQLKSANTGNNERIINVSIKKLKRKPPSTNATRRQKHRLTCPSCDSYEKKPPKEFLERFKSLLQKMIHQHLSSRTHGSEDS

SEQ ID NO: 91 - protein, 133 aa, Artificial
  Synthetic sequence
QGQDRHMIRMRQLIDIVDQLKNYVNDLVPEFLPAPEDVETNCEWSAFSCFQKAQLKSANTGNNERIINVSIKKLKRKPPSTNAGRRQKHRLTCPSCDSYEKKPPKEFLERFKSLLQKMINQTLSSRTHGSEDS

SEQ ID NO: 92 - protein, 133 aa, Artificial
  Synthetic sequence
QGQDRHMIRMRQLIDIVDQLKNYVNDLVPEFLPAPENVTTNCEWSAFSCFQKAQLKSANTGNNERIINVSIKKLKRKPPSTNAGRRQKHRLTCPSCDSYEKKPPKEFLERFKSLLQKMIHQHLSSRTHGSEDS

SEQ ID NO: 93 - protein, 133 aa, Artificial
  Synthetic sequence
QGQDRHMIRMRQLIDIVDQLKNYVNDLVPEFLPAPEDVETNCEWSAFSCFQKAQLKSANTGNNERIINVSIEKLKRKPPSTNAGRRQKHRLTCPSCDSYEKKPPKEFLERFKSLLQKMIHQHLSSRTHGSEDS

SEQ ID NO: 94 - protein, 133 aa, Artificial
  Synthetic sequence
QGQDRHMQRMRQLIDIVDQLKNYVNDLVPEFLPAPEDVETNCEWSAFSCFQKAQLKSANTGNNERIINVSIKKLKRKPESTNAGRRQKHRLTCPSCDSYEKKPPKEFLERFKSLLQKMIHQHLSSRTHGSEDS

SEQ ID NO: 95 - protein, 133 aa, Artificial
  Synthetic sequence
QGQDRHMIRMRQLIDIVDQLKNYVNDLVPEFLPAPEDVETNCEWSAFSCFQKAQLKSANTGNNERIINVSIKKLKRDAPSTNAGRRQKHRLTCPSCDSYEKKPPKEFLERFKSLLQKMIHQHLSSRTHGSEDS

SEQ ID NO: 96 - protein, 130 aa, Artificial
  Synthetic sequence
QGQDRHMIRMRQLIDIVDQLKNYVNDLVPEFLPAPEDVETNCEWSAFSCFQKAQLKSANTGNNERIINVSIKKLKRKPPSTNAGKHRLTCPSCDSYEKKPPKEFLERFKSLLQKMIHQHLSSRTHGSEDS

SEQ ID NO: 97 - protein, 131 aa, Artificial
  Synthetic sequence
QGQDRHMIRMRQLIDIVDQLKNYVNDLVPEFLPAPEDVETNCEWSAFSCFQKAQLKSANTGNNERIINVSIKKLKRKSTNAGRRQKHRLTCPSCDSYEKKPPKEFLERFKSLLQKMIHQHLSSRTHGSEDS

SEQ ID NO: 98 - protein, 124 aa, Artificial
  Synthetic sequence
MRQLIDIVDQLKNYVNDLVPEFLPAPEDVETNCEWSAFSCFQKAQLKSANTGNNERIINVSIKKLKRKPPSTNAGRRQKHRLTCPSCDSYEKKPPKEFLERFKSLLQKMIHQHLSSRTHGSEDS

SEQ ID NO: 99 - protein, 122 aa, Artificial
  Synthetic sequence
MRQLIDIVDQLKNYVNDLVPEFLPAPEDVETNCEWSAFSCFQKAQLKSANTGNNERIINVSIKKLKRKSTNAGRRQKHRLTCPSCDSYEKKPPKEFLERFKSLLQKMIHQHLSSRTHGSEDS

SEQ ID NO: 100 - protein, 124 aa, Artificial
  Synthetic sequence
MRQLIDIVDNLTNYVNDLVPEFLPAPEDVETNCEWSAFSCFQKAQLKSANTGNNERIINVSIKKLKRKPPSTNAGRRQKHRLTCPSCDSYEKKPPKEFLERFKSLLQKMIHQHLSSRTHGSEDS

SEQ ID NO: 101 - protein, 125 aa, Artificial
  Synthetic sequence
QGQDRHMIRMRQLIDIVDNLTNYVNDLVPEFLPAPEDVETNAEWSAFSCFQKAQLKSANTGNNERIINVSIKKLKRKPPSTNATTPSCDSYEKKPPKEFLERFKSLLQKMIHQHLSSRTHGSEDS

SEQ ID NO: 102 - protein, 131 aa, Artificial
  Synthetic sequence
HKSDITLQEMRQLIDIVDQLKNYVNDLVPEFLPAPEDVETNCEWSAFSCFQKAQLKSANTGNNERIINVSIKKLKRKSTNAGRRQKHRLTCPSCDSYEKKPPKEFLERFKSLLQKMIHQHLSSRTHGSEDS

SEQ ID NO: 103 - protein, 133 aa, Artificial
  Synthetic sequence
HKSDITLQEMRQLIDIVDQLKNYVNDLVPEFLPAPEDVETNCEWSAFSCFQKAQLKSANTGNNERIINVSIKKLKRKPPSTNAGRRQKHRLTCPSCDSYEKKPPKEFLERFKSLLQNMTHQHLSSRTHGSEDS

SEQ ID NO: 104 - protein, 133 aa, Artificial
  Synthetic sequence
HKSDITLQEMRQLIDIVDQLKNYVNDLVPEFLPAPENVTTNCEWSAFSCFQKAQLKSANTGNNERIINVSIKKLKRKPPSTNAGRRQKHRLTCPSCDSYEKKPPKEFLERFKSLLQKMIHQHLSSRTHGSEDS

SEQ ID NO: 105 - protein, 133 aa, Artificial
  Synthetic sequence
HKSDITLQEMRQLINITDQLKNYVNDLVPEFLPAPEDVETNCEWSAFSCFQKAQLKSANTGNNERIINVSIKKLKRKPPSTNAGRRQKHRLTCPSCDSYEKKPPKEFLERFKSLLQKMIHQHLSSRTHGSEDS

SEQ ID NO: 106 - protein, 161 aa, Homo sapiens
  IL-21wt including signal peptide
MRSSPGNMERIVICLMVIFLGTLVHKSSSQGQDRHMIRMRQLIDIVDQLKNYVNDLVPEFLPAPEDVETNEWSAFSCFQKAQLKSANTGNNERIINVSIKKLKRKPPSTNAGRRQKHRLTCPSCDSYEKKPPKEFLERFKSLLQKMIHQHLSSRTHGSEDS

SEQ ID NO: 107 - protein, 153 aa, Homo sapiens
  IL-21 natural variant
MRSSPGNMERIVICLMVIFLGTLVHKSSSQGQDRHMIRMRQLIDIVDQLKNYVNDLVPEFLPAPEDVETNCEWSAFSCFQKAQLKSANTGNNERIINVSIKKLKRKPPSTNAGRRQKHRLTCPSCDSYEKKPPKEFLERFKSLLQKVSTLSFI

SEQ ID NO: 108 - protein, 124 aa, Homo sapiens
  IL-21 natural variant comrising signal peptide
QGQDRHMIRMRQLIDIVDQLKNYVNDLVPEFLPAPEDVETNCEWSAFSCFQKAQLKSANTGNNERIINVSIKKLKRKPPSTNAGRRQKHRLTCPSCDSYEKKPPKEFLERFKSLLQKVSTLSFI

SEQ ID NO: 109 - protein, 13 aa, Artificial
  Synthetic sequence
KASGGTFSSYAIS

SEQ ID NO: 110 - protein, 17 aa, Artificial
  Synthetic sequence
LIIPMFDTAGYAQKFQG

SEQ ID NO: 111 - protein, 13 aa, Artificial
  Synthetic sequence
ARAEHSSTGTFDY

SEQ ID NO: 112 - protein, 11 aa, Artificial
  Synthetic sequence
RASQGISSWLA

SEQ ID NO: 113 - protein, 8 aa, Artificial
  Synthetic sequence
SAASSLQS

SEQ ID NO: 114 - protein, 9 aa, Artificial
  Synthetic sequence
QQANHLPFT

SEQ ID NO: 115 - protein, 120 aa, Artificial
  Synthetic sequence
QVQLVQSGAEVKKPGSSVKVSCKASGGTFSSYAISWVRQAPGQGLEWMGLIIPMFDTAGYAQKFQGRVAITVDESTSTAYMELSSLRSEDTAVYYCARAEHSSTGTFDYWGQGTLVTVSS

SEQ ID NO: 116 - protein, 107 aa, Artificial
  Synthetic sequence
DIQMTQSPSSVSASVGDRVTITCRASQGISSWLAWYQQKPGKAPKLLISAASSLQSGVPSRFSGSGSGTDFTLTISSLQPEDFATYYCQQANHLPFTFGGGTKVEIK

SEQ ID NO: 117 - protein, 129 aa, Artificial [sequence omitted]